European Patent Application EP 4 574 966 A1, published June 25, 2025. Title: ENGINEERED CELL LINES FOR THE PRODUCTION OF CULTIVATED MEAT. Applicant: GOOD Meat, Inc. Application EP, filed December 18, 2024. The sequence listing filed with the application follows.

SEQUENCE LISTING (10 sequences)

SEQ ID NO: 1 - RNA, 20 nt, synthetic construct
  source 1..20: mol_type = other RNA
caaccacgctgatcttgttg

SEQ ID NO: 2 - RNA, 20 nt, synthetic construct
  source 1..20: mol_type = other RNA
ggtgttctgagaagattgtc

SEQ ID NO: 3 - RNA, 23 nt, synthetic construct
  source 1..23: mol_type = other RNA
caaccacgctgatcttgttgtgg

SEQ ID NO: 4 - RNA, 23 nt, synthetic construct
  source 1..23: mol_type = other RNA
ggtgttctgagaagattgtctgg

SEQ ID NO: 5 - DNA, 87 bp, Gallus gallus
  source 1..87: mol_type = genomic DNA
ctcatccacaatgtccacaaagaggagcacgctcatgcccacaacaagatcagcgtggttggtgtgggtgcagttggaatggcttgt

SEQ ID NO: 6 - DNA, 87 bp, Gallus gallus
  source 1..87: mol_type = genomic DNA
taagattagcaaacataatgaaggaaataagtctgcttccagacaatcttctcagaacaccttcagttcagctggtgcagagttggt

SEQ ID NO: 7 - DNA, 73 bp, synthetic construct
  source 1..73: mol_type = other DNA
aagaggagcacgctcatgcccacaaagatcagcgtggttggtgtgggtgcagttggaatggcttgtgccatca

SEQ ID NO: 8 - DNA, 71 bp, synthetic construct
  source 1..71: mol_type = other DNA
gaactgaaggtgttctgagaagattggaagcagacttatttccttcattatgtttgctaatcttacaggca

SEQ ID NO: 9 - DNA, 73 bp, synthetic construct
  source 1..73: mol_type = other DNA
gaactgaaggtgttctgagaagagtctggaagcagacttatttccttcattatgtttgctaatcttacaggca

SEQ ID NO: 10 - DNA, 73 bp, synthetic construct
  source 1..73: mol_type = other DNA
gaactgaaggtgttctgagaagattctggaagcagacttatttccttcattatgtttgctaatcttacaggca